European Patent Specification EP 3 615 674 B1, published March 13, 2024. Title: Methods of Treating Rheumatoid Arthritis Using RNA-Guided Genome Editing of HLA Gene. Applicant: The Regents of the University of Colorado, a body corporate Freed, Brian Roark, Christina Anderson, Kirsten Matsuda, Jennifer. Application Not yet assigned. The sequence listing filed with the application follows.

SEQUENCE LISTING (3 sequences)

SEQ ID NO: 1 - RNA, 23 nt, Artificial Sequence
  Synthetic Guide Sequence
ggaccucgucuucgcccggcgcc

SEQ ID NO: 2 - DNA, 20 bp, Artificial Sequence
  Synthetic Guide Sequence
cggcccgcttctgctccagg

SEQ ID NO: 3 - DNA, 20 bp, Artificial Sequence
  Synthetic Guide Sequence
cctggagcagaagcgggccg